European Patent Application EP 4 368 710 A1, published May 15, 2024. Title: LINEAR PEPTIDES INHIBITING CK2-MEDIATED PHOSPHORYLATION AND COMPOSITIONS COMPRISING THEREOF. Applicant: CENTRO DE INGENIERIA GENETICA Y BIOTECNOLOGIA. Application CU. The sequence listing filed with the application follows.

SEQUENCE LISTING (66 sequences)

SEQ ID NO: 1 - protein, 8 aa, synthetic construct
  REGION 1..8: note = Description of the artificial sequence: linear peptide
RLRRKADP

SEQ ID NO: 2 - protein, 8 aa, synthetic construct
  REGION 1..8: note = Description of the artificial sequence: Linear peptide
LRRRKADP

SEQ ID NO: 3 - protein, 8 aa, synthetic construct
  REGION 1..8: note = Description of the artificial sequence: Linear peptide
TYRYRRDP

SEQ ID NO: 4 - protein, 8 aa, synthetic construct
  REGION 1..8: note = Description of the artificial sequence: Linear peptide
VARRRYDP

SEQ ID NO: 5 - protein, 8 aa, synthetic construct
  REGION 1..8: note = Description of the artificial sequence: Linear peptide
AVRRRYDP

SEQ ID NO: 6 - protein, 8 aa, synthetic construct
  REGION 1..8: note = Description of the artificial sequence: Linear peptide
TFYRRYDP

SEQ ID NO: 7 - protein, 8 aa, synthetic construct
  REGION 1..8: note = Description of the artificial sequence: Linear peptide
RKRSRYDP

SEQ ID NO: 8 - protein, 8 aa, synthetic construct
  REGION 1..8: note = Description of the artificial sequence: Linear peptide
GYRYKRDP

SEQ ID NO: 9 - protein, 8 aa, synthetic construct
  REGION 1..8: note = Description of the artificial sequence: Linear peptide
VKKRRLDP

SEQ ID NO: 10 - protein, 8 aa, synthetic construct
  REGION 1..8: note = Description of the artificial sequence: Linear peptide
EQPAFHDP

SEQ ID NO: 11 - protein, 8 aa, synthetic construct
  REGION 1..8: note = Description of the artificial sequence: Linear peptide
VAGFFLDP

SEQ ID NO: 12 - protein, 22 aa, synthetic construct
  REGION 1..22: note = Description of the artificial sequence: Linear polypeptide
  MOD_RES 14: note = bAla
GRKKRRQRRRPPQARLRRKADP

SEQ ID NO: 13 - protein, 22 aa, synthetic construct
  REGION 1..22: note = Description of the artificial sequence: Linear polypeptide
  MOD_RES 14: note = bAla
GRKKRRQRRRPPQALRRRKADP

SEQ ID NO: 14 - protein, 22 aa, synthetic construct
  REGION 1..22: note = Description of the artificial sequence: Linear polypeptide
  MOD_RES 14: note = bAla
GRKKRRQRRRPPQATYRYRRDP

SEQ ID NO: 15 - protein, 22 aa, synthetic construct
  REGION 1..22: note = Description of the artificial sequence: Linear polypeptide
  MOD_RES 14: note = bAla
GRKKRRQRRRPPQAVARRRYDP

SEQ ID NO: 16 - protein, 22 aa, synthetic construct
  REGION 1..22: note = Description of the artificial sequence: Linear polypeptide
  MOD_RES 14: note = bAla
GRKKRRQRRRPPQAAVRRRYDP

SEQ ID NO: 17 - protein, 22 aa, synthetic construct
  REGION 1..22: note = Description of the artificial sequence: Linear polypeptide
  MOD_RES 14: note = bAla
GRKKRRQRRRPPQATFYRRYDP

SEQ ID NO: 18 - protein, 22 aa, synthetic construct
  REGION 1..22: note = Description of the artificial sequence: Linear polypeptide
  MOD_RES 14: note = bAla
GRKKRRQRRRPPQARKRSRYDP

SEQ ID NO: 19 - protein, 22 aa, synthetic construct
  REGION 1..22: note = Description of the artificial sequence: Linear polypeptide
  MOD_RES 14: note = bAla
GRKKRRQRRRPPQAGYRYKRDP

SEQ ID NO: 20 - protein, 22 aa, synthetic construct
  REGION 1..22: note = Description of the artificial sequence: Linear polypeptide
  MOD_RES 14: note = bAla
GRKKRRQRRRPPQAVKKRRLDP

SEQ ID NO: 21 - protein, 22 aa, synthetic construct
  REGION 1..22: note = Description of the artificial sequence: Trp-scanning polypeptide
  MOD_RES 14: note = bAla
GRKKRRQRRRPPQAWYRYKRDP

SEQ ID NO: 22 - protein, 22 aa, synthetic construct
  REGION 1..22: note = Description of the artificial sequence: Trp scanning polypeptide
  MOD_RES 14: note = bAla
GRKKRRQRRRPPQAGWRYKRDP

SEQ ID NO: 23 - protein, 22 aa, synthetic construct
  REGION 1..22: note = Description of the artificial sequence: Trp scanning polypeptide
  MOD_RES 14: note = bAla
GRKKRRQRRRPPQAGYWYKRDP

SEQ ID NO: 24 - protein, 22 aa, synthetic construct
  REGION 1..22: note = Description of the artificial sequence: Trp scanning polypeptide
  MOD_RES 14: note = bAla
GRKKRRQRRRPPQAGYRWKRDP

SEQ ID NO: 25 - protein, 22 aa, synthetic construct
  REGION 1..22: note = Description of the artificial sequence: Trp scanning polypeptide
  MOD_RES 14: note = bAla
GRKKRRQRRRPPQAGYRYWRDP

SEQ ID NO: 26 - protein, 22 aa, synthetic construct
  REGION 1..22: note = Description of the artificial sequence: Trp scanning polypeptide
  MOD_RES 14: note = bAla
GRKKRRQRRRPPQAGYRYKWDP

SEQ ID NO: 27 - protein, 22 aa, synthetic construct
  REGION 1..22: note = Description of the artificial sequence: Trp scanning polypeptide
  MOD_RES 14: note = bAla
GRKKRRQRRRPPQAGYRYKRWP

SEQ ID NO: 28 - protein, 22 aa, synthetic construct
  REGION 1..22: note = Description of the artificial sequence: Trp scanning polypeptide
  MOD_RES 14: note = bAla
GRKKRRQRRRPPQAGYRYKRDW

SEQ ID NO: 29 - protein, 22 aa, synthetic construct
  REGION 1..22: note = Description of the artificial sequence: Trp scanning polypeptide
  MOD_RES 14: note = bAla
GRKKRRQRRRPPQAWKRSRYDP

SEQ ID NO: 30 - protein, 22 aa, synthetic construct
  REGION 1..22: note = Description of the artificial sequence: Trp scanning polypeptide
  MOD_RES 14: note = bAla
GRKKRRQRRRPPQARWRSRYDP

SEQ ID NO: 31 - protein, 22 aa, synthetic construct
  REGION 1..22: note = Description of the artificial sequence: Trp scanning polypeptide
  MOD_RES 14: note = bAla
GRKKRRQRRRPPQARKWSRYDP

SEQ ID NO: 32 - protein, 22 aa, synthetic construct
  REGION 1..22: note = Description of the artificial sequence: Trp scanning polypeptide
  MOD_RES 14: note = bAla
GRKKRRQRRRPPQARKRWRYDP

SEQ ID NO: 33 - protein, 22 aa, synthetic construct
  REGION 1..22: note = Description of the artificial sequence: Trp scanning polypeptide
  MOD_RES 14: note = bAla
GRKKRRQRRRPPQARKRSWYDP

SEQ ID NO: 34 - protein, 22 aa, synthetic construct
  REGION 1..22: note = Description of the artificial sequence: Trp scanning polypeptide
  MOD_RES 14: note = bAla
GRKKRRQRRRPPQARKRSRWDP

SEQ ID NO: 35 - protein, 22 aa, synthetic construct
  REGION 1..22: note = Description of the artificial sequence: Trp scanning polypeptide
  MOD_RES 14: note = bAla
GRKKRRQRRRPPQARKRSRYWP

SEQ ID NO: 36 - protein, 22 aa, synthetic construct
  REGION 1..22: note = Description of the artificial sequence: Trp scanning polypeptide
  MOD_RES 14: note = bAla
GRKKRRQRRRPPQARKRSRYDW

SEQ ID NO: 37 - protein, 22 aa, synthetic construct
  REGION 1..22: note = Description of the artificial sequence: Trp scanning polypeptide
  MOD_RES 14: note = bAla
GRKKRRQRRRPPQAWKKRRLDP

SEQ ID NO: 38 - protein, 22 aa, synthetic construct
  REGION 1..22: note = Description of the artificial sequence: Trp scanning polypeptide
  MOD_RES 14: note = bAla
GRKKRRQRRRPPQAVWKRRLDP

SEQ ID NO: 39 - protein, 22 aa, synthetic construct
  REGION 1..22: note = Description of the artificial sequence: Trp scanning polypeptide
  MOD_RES 14: note = bAla
GRKKRRQRRRPPQAVKWRRLDP

SEQ ID NO: 40 - protein, 22 aa, synthetic construct
  REGION 1..22: note = Description of the artificial sequence: Trp scanning polypeptide
  MOD_RES 14: note = bAla
GRKKRRQRRRPPQAVKKWRLDP

SEQ ID NO: 41 - protein, 22 aa, synthetic construct
  REGION 1..22: note = Description of the artificial sequence: Trp scanning polypeptide
  MOD_RES 14: note = bAla
GRKKRRQRRRPPQAVKKRWLDP

SEQ ID NO: 42 - protein, 22 aa, synthetic construct
  REGION 1..22: note = Description of the artificial sequence: Trp scanning polypeptide
  MOD_RES 14: note = bAla
GRKKRRQRRRPPQAVKKRRWDP

SEQ ID NO: 43 - protein, 22 aa, synthetic construct
  REGION 1..22: note = Description of the artificial sequence: Trp scanning polypeptide
  MOD_RES 14: note = bAla
GRKKRRQRRRPPQAVKKRRLWP

SEQ ID NO: 44 - protein, 22 aa, synthetic construct
  REGION 1..22: note = Description of the artificial sequence: Trp scanning polypeptide
  MOD_RES 14: note = bAla
GRKKRRQRRRPPQAVKKRRLDW

SEQ ID NO: 45 - protein, 8 aa, synthetic construct
  REGION 1..8: note = Description of the artificial sequence: modified linear peptide
RKRSRYWP

SEQ ID NO: 46 - protein, 22 aa, synthetic construct
  REGION 1..22: note = Description of the artificial sequence: Modified linear polypeptide
  MOD_RES 14: note = bAla
GRKKRRQRRRPPQAWKRSRYWP

SEQ ID NO: 47 - protein, 22 aa, synthetic construct
  REGION 1..22: note = Description of the artificial sequence: Modified linear polypeptide
  MOD_RES 14: note = bAla
GRKKRRQRRRPPQARKRWRYWP

SEQ ID NO: 48 - protein, 22 aa, synthetic construct
  REGION 1..22: note = Description of the artificial sequence: Modified linear polypeptide
  MOD_RES 14: note = bAla
GRKKRRQRRRPPQARKRSWYWP

SEQ ID NO: 49 - protein, 8 aa, synthetic construct
  REGION 1..8: note = Description of the artificial sequence: modified linear peptide
RKRWRYWP

SEQ ID NO: 50 - protein, 8 aa, synthetic construct
  REGION 1..8: note = Description of the artificial sequence: modified linear peptide
RKRSWYWP

SEQ ID NO: 51 - protein, 22 aa, synthetic construct
  REGION 1..22: note = Description of the artificial sequence: Modified linear polypeptide where Arg 8 and Lys16 are D a.a
  MOD_RES 1: note = ACETYLATION
  MOD_RES 14: note = bAla
GRKKRRQRRRPPQARKRWRYWP

SEQ ID NO: 52 - protein, 22 aa, synthetic construct
  REGION 1..22: note = Description of the artificial sequence: modified linear polypeptide where Arg 8 and Arg 17 are D a.a.
  MOD_RES 1: note = ACETYLATION
  MOD_RES 14: note = bAla
GRKKRRQRRRPPQARKRWRYWP

SEQ ID NO: 53 - protein, 22 aa, synthetic construct
  REGION 1..22: note = Description of the artificial sequence: Modified linear polypeptide where Arg 8 is a D a.a. and Tyr 20 is NMeTyr
  MOD_RES 1: note = ACETYLATION
  MOD_RES 14: note = bAla
GRKKRRQRRRPPQARKRWRYWP

SEQ ID NO: 54 - protein, 22 aa, synthetic construct
  REGION 1..22: note = Description of the artificial sequence: Modified linear polypeptide where Arg 8 and Lys 16 are D a.a.
  MOD_RES 1: note = ACETYLATION
  MOD_RES 14: note = bAla
GRKKRRQRRRPPQARKRSWYWP

SEQ ID NO: 55 - protein, 22 aa, synthetic construct
  REGION 1..22: note = Description of the artificial sequence: Modified linear polypeptide where Arg 8 and Arg 17 are D a.a.
  MOD_RES 1: note = ACETYLATION
  MOD_RES 14: note = bAla
GRKKRRQRRRPPQARKRSWYWP

SEQ ID NO: 56 - protein, 22 aa, synthetic construct
  REGION 1..22: note = Description of the artificial sequence: Modified linear polypeptide where Arg 8 is a Da.a. and Tyr 20 is NMe Tyr
  MOD_RES 1: note = ACETYLATION
  MOD_RES 14: note = bAla
GRKKRRQRRRPPQARKRSWYWP

SEQ ID NO: 57 - protein, 8 aa, synthetic construct
  REGION 1..8: note = Description of the artificial sequence: Modified linear peptide where Lys 2 is a D a.a.
RKRWRYWP

SEQ ID NO: 58 - protein, 8 aa, synthetic construct
  REGION 1..8: note = Description of the artificial sequence: Modified linear peptide where Arg 3 is a D a.a.
RKRWRYWP

SEQ ID NO: 59 - protein, 8 aa, synthetic construct
  REGION 1..8: note = Description of the artificial sequence: Modified linear peptide where Tyr 6 is NMe Tyr
RKRWRYWP

SEQ ID NO: 60 - protein, 8 aa, synthetic construct
  REGION 1..8: note = Description of the artificial sequence: Modified linear peptide where Lys 2 is a D a.a.
RKRSWYWP

SEQ ID NO: 61 - protein, 8 aa, synthetic construct
  REGION 1..8: note = Description of the artificial sequence: Modified linear peptide where Arg 3 is a D a.a.
RKRSWYWP

SEQ ID NO: 62 - protein, 8 aa, synthetic construct
  REGION 1..8: note = Description of the artificial sequence: Modified linear peptide where Tyr 6 is NMe Tyr
RKRSWYWP

SEQ ID NO: 63 - protein, 11 aa, human papilloma virus type 16
LNDSSEEEDEI

SEQ ID NO: 64 - protein, 25 aa, synthetic construct
  REGION 1..25: note = Description of the artificial sequence: Modified peptide where Cys 15 and Cys 25 form a cycle
  MOD_RES 14: note = bAla
GRKKRRQRRRPPQACWMSPRHLGTC

SEQ ID NO: 65 - protein, 13 aa, Human immunodeficiency virus type 1
GRKKRRQRRRPPQ

SEQ ID NO: 66 - protein, 13 aa, synthetic construct
  REGION 1..13: note = Description of the artificial sequence: Modified linear peptide where Arg 8 is a D a.a.
GRKKRRQRRRPPQ